European Patent Specification EP 4 404 956 B1, published April 1, 2026. Title: Binding Proteins for Terminal Deoxynucleotidyl Transferase (TdT). Applicant: Oslo universitetssykehus HF. The sequence listing filed with the application follows.

SEQUENCE LISTING (55 sequences)

SEQ ID NO: 1 - protein, 9 aa, unidentified
ALYDKTKRI

SEQ ID NO: 2 - protein, 6 aa, unidentified
VSGLRG

SEQ ID NO: 3 - protein, 7 aa, unidentified
LYSAGEE

SEQ ID NO: 4 - protein, 15 aa, unidentified
CAVQASSNSGYALNF

SEQ ID NO: 5 - protein, 5 aa, unidentified
SQVTM

SEQ ID NO: 6 - protein, 7 aa, unidentified
ANQGSEA

SEQ ID NO: 7 - protein, 13 aa, unidentified
CSVEPGYADTQYF

SEQ ID NO: 8 - protein, 111 aa, unidentified
EDQVTQSPEALRLQEGESSSLNCSYTVSGLRGLFWYRQDPGKGPEFLFTLYSAGEEKEKERLKATLTKKESFLHITAPKPEDSATYLCAVQASSNSGYALNFGKGTSLLVT

SEQ ID NO: 9 - protein, 114 aa, unidentified
SAVISQKPSRDICQRGTSLTIQCQVDSQVTMMFWYRQQPGQSLTLIATANQGSEATYESGFVIDKFPISRPNLTFSTLTVSNMSPEDSSIYLCSVEPGYADTQYFGPGTRLTVL

SEQ ID NO: 10 - protein, 108 aa, unidentified
PDIQNPEPAVYQLKDPRSQDSTLCLFTDFDSQINVPKTMESGTFITDKCVLDMKAMDSKSNGAIAWSNQTSFTCQDIFKETNATYPSSDVPCDATLTEKSFETDMNLN

SEQ ID NO: 11 - protein, 140 aa, unidentified
EDLRNVTPPKVSLFEPSKAEIANKQKATLVCLARGFFPDHVELSWWVNGKEVHSGVCTDPQAYKESNYSYCLSSRLRVSATFWHNPRNHFRCQVQFHGLSEEDKWPEGSPKPVTQNISAEAWGRADCGITSASYHQGVLS

SEQ ID NO: 12 - protein, 249 aa, unidentified
EDQVTQSPEALRLQEGESSSLNCSYTVSGLRGLFWYRQDPGKGPEFLFTLYSAGEEKEKERLKATLTKKESFLHITAPKPEDSATYLCAVQASSNSGYALNFGKGTSLLVTPDIQNPEPAVYQLKDPRSQDSTLCLFTDFDSQINVPKTMESGTFITDKCVLDMKAMDSKSNGAIAWSNQTSFTCQDIFKETNATYPSSDVPCDATLTEKSFETDMNLNFQNLSVMGLRILLLKVAGFNLLMTLRLWSS

SEQ ID NO: 13 - protein, 287 aa, unidentified
SAVISQKPSRDICQRGTSLTIQCQVDSQVTMMFWYRQQPGQSLTLIATANQGSEATYESGFVIDKFPISRPNLTFSTLTVSNMSPEDSSIYLCSVEPGYADTQYFGPGTRLTVLEDLRNVTPPKVSLFEPSKAEIANKQKATLVCLARGFFPDHVELSWWVNGKEVHSGVCTDPQAYKESNYSYCLSSRLRVSATFWHNPRNHFRCQVQFHGLSEEDKWPEGSPKPVTQNISAEAWGRADCGITSASYHQGVLSATILYEILLGKATLYAVLVSGLVLMAMVKKKNS

SEQ ID NO: 14 - protein, 594 aa, unidentified
MLSLLLLLLGLGSVFSAVISQKPSRDICQRGTSLTIQCQVDSQVTMMFWYRQQPGQSLTLIATANQGSEATYESGFVIDKFPISRPNLTFSTLTVSNMSPEDSSIYLCSVEPGYADTQYFGPGTRLTVLEDLRNVTPPKVSLFEPSKAEIANKQKATLVCLARGFFPDHVELSWWVNGKEVHSGVCTDPQAYKESNYSYCLSSRLRVSATFWHNPRNHFRCQVQFHGLSEEDKWPEGSPKPVTQNISAEAWGRADCGITSASYHQGVLSATILYEILLGKATLYAVLVSGLVLMAMVKKKNSGSGATNFSLLKQAGDVEENPGPMKSLRVLLVILWLQLSWVWSQEDQVTQSPEALRLQEGESSSLNCSYTVSGLRGLFWYRQDPGKGPEFLFTLYSAGEEKEKERLKATLTKKESFLHITAPKPEDSATYLCAVQASSNSGYALNFGKGTSLLVTPDIQNPEPAVYQLKDPRSQDSTLCLFTDFDSQINVPKTMESGTFITDKCVLDMKAMDSKSNGAIAWSNQTSFTCQDIFKETNATYPSSDVPCDATLTEKSFETDMNLNFQNLSVMGLRILLLKVAGFNLLMTLRLWSS

SEQ ID NO: 15 - protein, 11 aa, unidentified
ALYDKTKRIFL

SEQ ID NO: 16 - protein, 5 aa, unidentified
TSINN

SEQ ID NO: 17 - protein, 7 aa, unidentified
IRSNERE

SEQ ID NO: 18 - protein, 18 aa, unidentified
CATDAGAYSGGGADGLTF

SEQ ID NO: 19 - protein, 5 aa, unidentified
MNHEY

SEQ ID NO: 20 - protein, 6 aa, unidentified
SMNVEV

SEQ ID NO: 21 - protein, 14 aa, unidentified
CASSLSSSYNEQFF

SEQ ID NO: 22 - protein, 115 aa, unidentified
SQQGEEDPQALSIQEGENATMNCSYKTSINNLQWYRQNSGRGLVHLILIRSNEREKHSGRLRVTLDTSKKSSSLLITASRAADTASYFCATDAGAYSGGGADGLTFGKGTHLIIQ

SEQ ID NO: 23 - protein, 113 aa, unidentified
EAQVTQNPRYLITVTGKKLTVTCSQNMNHEYMSWYRQDPGLGLRQIYYSMNVEVTDKGDVPEGYKVSRKEKRNFPLILESPSPNQTSLYFCASSLSSSYNEQFFGPGTRLTVL

SEQ ID NO: 24 - protein, 253 aa, unidentified
SQQGEEDPQALSIQEGENATMNCSYKTSINNLQWYRQNSGRGLVHLILIRSNEREKHSGRLRVTLDTSKKSSSLLITASRAADTASYFCATDAGAYSGGGADGLTFGKGTHLIIQPDIQNPEPAVYQLKDPRSQDSTLCLFTDFDSQINVPKTMESGTFITDKCVLDMKAMDSKSNGAIAWSNQTSFTCQDIFKETNATYPSSDVPCDATLTEKSFETDMNLNFQNLSVMGLRILLLKVAGFNLLMTLRLWSS

SEQ ID NO: 25 - protein, 286 aa, unidentified
EAQVTQNPRYLITVTGKKLTVTCSQNMNHEYMSWYRQDPGLGLRQIYYSMNVEVTDKGDVPEGYKVSRKEKRNFPLILESPSPNQTSLYFCASSLSSSYNEQFFGPGTRLTVLEDLRNVTPPKVSLFEPSKAEIANKQKATLVCLARGFFPDHVELSWWVNGKEVHSGVCTDPQAYKESNYSYCLSSRLRVSATFWHNPRNHFRCQVQFHGLSEEDKWPEGSPKPVTQNISAEAWGRADCGITSASYHQGVLSATILYEILLGKATLYAVLVSGLVLMAMVKKKNS

SEQ ID NO: 26 - protein, 22 aa, Porcine Teschovirus
GSGATNFSLLKQAGDVEENPGP

SEQ ID NO: 27 - protein, 509 aa, Homo sapiens
MDPPRASHLSPRKKRPRQTGALMASSPQDIKFQDLVVFILEKKMGTTRRAFLMELARRKGFRVENELSDSVTHIVAENNSGSDVLEWLQAQKVQVSSQPELLDVSWLIECIRAGKPVEMTGKHQLVVRRDYSDSTNPGPPKTPPIAVQKISQYACQRRTTLNNCNQIFTDAFDILAENCEFRENEDSCVTFMRAASVLKSLPFTIISMKDTEGIPCLGSKVKGIIEEIIEDGESSEVKAVLNDERYQSFKLFTSVFGVGLKTSEKWFRMGFRTLSKVRSDKSLKFTRMQKAGFLYYEDLVSCVTRAEAEAVSVLVKEAVWAFLPDAFVTMTGGFRRGKKMGHDVDFLITSPGSTEDEEQLLQKVMNLWEKKGLLLYYDLVESTFEKLRLPSRKVDALDHFQKCFLIFKLPRQRVDSDQSSWQEGKTWKAIRVDLVLCPYERRAFALLGWTGSRQFERDLRRYATHERKMILDNHALYDKTKRIFLKAESEEEIFAHLGLDYIEPWERNA

SEQ ID NO: 28 - protein, 112 aa, Homo sapiens
PNIQNPDPAVYQLRDSKSSDKSVCLFTDFDSQTNVSQSKDSDVYITDKTVLDMRSMDFKSNSAVAWSNKSDFACANAFNNSIIPEDTFFPSPESSCDVKLVEKSFETDTNLN

SEQ ID NO: 29 - protein, 144 aa, Homo sapiens
EDLNKVFPPEVAVFEPSEAEISHTQKATLVCLATGFFPDHVELSWWVNGKEVHSGVSTDPQPLKEQPALNDSRYCLSSRLRVSATFWQNPRNHFRCQVQFYGLSENDEWTQDRAKPVTQIVSAEAWGRADCGFTSVSYQQGVLS

SEQ ID NO: 30 - protein, 144 aa, Homo sapiens
EDLKNVFPPKVAVFEPSEAEISHTQKATLVCLATGFYPDHVELSWWVNGKEVHSGVSTDPQPLKEQPALNDSRYCLSSRLRVSATFWQNPRNHFRCQVQFYGLSENDEWTQDRAKPVTQIVSAEAWGRADCGFTSESYQQGVLS

SEQ ID NO: 31 - protein, 108 aa, Mus musculus
PDIQNPEPAVYQLKDPRSQDSTLCLFTDFDSQINVPKTMESGTFITDKTVLDMKAMDSKSNGAIAWSNQTSFTCQDIFKETNATYPSSDVPCDATLTEKSFETDMNLN

SEQ ID NO: 32 - protein, 140 aa, Mus musculus
EDLRNVTPPKVSLFEPSKAEIANKQKATLVCLARGFFPDHVELSWWVNGKEVHSGVSTDPQAYKESNYSYCLSSRLRVSATFWHNPRNHFRCQVQFHGLSEEDKWPEGSPKPVTQNISAEAWGRADCGITSASYQQGVLS

SEQ ID NO: 33 - protein, 140 aa, Mus musculus
EDLRNVTPPKVSLFEPSKAEIANKQKATLVCLARGFFPDHVELSWWVNGKEVHSGVSTDPQAYKESNYSYCLSSRLRVSATFWHNPRNHFRCQVQFHGLSEEDKWPEGSPKPVTQNISAEAWGRADCGITSASYHQGVLS

SEQ ID NO: 34 - protein, 112 aa, Homo sapiens
PNIQNPDPAVYQLRDSKSSDKSVCLFTDFDSQTNVSQSKDSDVYITDKCVLDMRSMDFKSNSAVAWSNKSDFACANAFNNSIIPEDTFFPSPESSCDVKLVEKSFETDTNLN

SEQ ID NO: 35 - protein, 144 aa, Homo sapiens
EDLNKVFPPEVAVFEPSEAEISHTQKATLVCLATGFFPDHVELSWWVNGKEVHSGVCTDPQPLKEQPALNDSRYCLSSRLRVSATFWQNPRNHFRCQVQFYGLSENDEWTQDRAKPVTQIVSAEAWGRADCGFTSVSYQQGVLS

SEQ ID NO: 36 - protein, 144 aa, Homo sapiens
EDLKNVFPPKVAVFEPSEAEISHTQKATLVCLATGFYPDHVELSWWVNGKEVHSGVCTDPQPLKEQPALNDSRYCLSSRLRVSATFWQNPRNHFRCQVQFYGLSENDEWTQDRAKPVTQIVSAEAWGRADCGFTSESYQQGVLS

SEQ ID NO: 37 - protein, 140 aa, Mus musculus
EDLRNVTPPKVSLFEPSKAEIANKQKATLVCLARGFFPDHVELSWWVNGKEVHSGVCTDPQAYKESNYSYCLSSRLRVSATFWHNPRNHFRCQVQFHGLSEEDKWPEGSPKPVTQNISAEAWGRADCGITSASYQQGVLS

SEQ ID NO: 38 - protein, 25 aa, Homo sapiens
FQNLSVIGFRILLLKVAGFNLLMTL

SEQ ID NO: 39 - protein, 18 aa, Homo Sapiens/Mus Musculus
ATILYEILLGKATLYAVL

SEQ ID NO: 40 - protein, 27 aa, Homo sapiens
FWVLVVVGGVLACYSLLVTVAFIIFWV

SEQ ID NO: 41 - protein, 5 aa, Homo Sapiens/Mus Musculus
RLWSS

SEQ ID NO: 42 - protein, 15 aa, Homo sapiens
VSALVLMAMVKRKDF

SEQ ID NO: 43 - protein, 17 aa, Homo sapiens
VSALVLMAMVKRKDSRG

SEQ ID NO: 44 - protein, 25 aa, Mus musculus
FQNLSVMGLRILLLKVAGFNLLMTL

SEQ ID NO: 45 - protein, 601 aa, unidentified
MGPQLLGYVVLCLLGAGPLEAQVTQNPRYLITVTGKKLTVTCSQNMNHEYMSWYRQDPGLGLRQIYYSMNVEVTDKGDVPEGYKVSRKEKRNFPLILESPSPNQTSLYFCASSLSSSYNEQFFGPGTRLTVLEDLRNVTPPKVSLFEPSKAEIANKQKATLVCLARGFFPDHVELSWWVNGKEVHSGVCTDPQAYKESNYSYCLSSRLRVSATFWHNPRNHFRCQVQFHGLSEEDKWPEGSPKPVTQNISAEAWGRADCGITSASYHQGVLSATILYEILLGKATLYAVLVSGLVLMAMVKKKNSGSGATNFSLLKQAGDVEENPGPMKSLRVLLVILWLQLSWVWSQSQQGEEDPQALSIQEGENATMNCSYKTSINNLQWYRQNSGRGLVHLILIRSNEREKHSGRLRVTLDTSKKSSSLLITASRAADTASYFCATDAGAYSGGGADGLTFGKGTHLIIQPDIQNPEPAVYQLKDPRSQDSTLCLFTDFDSQINVPKTMESGTFITDKCVLDMKAMDSKSNGAIAWSNQTSFTCQDIFKETNATYPSSDVPCDATLTEKSFETDMNLNFQNLSVMGLRILLLKVAGFNLLMTLRLWSS

SEQ ID NO: 46 - protein, 15 aa, Mus musculus
VSTLVVMAMVKRKNS

SEQ ID NO: 47 - protein, 15 aa, Mus musculus
VSGLVLMAMVKKKNS

SEQ ID NO: 48 - protein, 112 aa, Homo sapiens
RVKFSRSADAPAYQQGQNQLYNELNLGRREEYDVLDKRRGRDPEMGGKPRRKNPQEGLYNELQKDKMAEAYSEIGMKGERRRGKGHDGLYQGLSTATKDTYDALHMQALPPR

SEQ ID NO: 49 - protein, 41 aa, Homo sapiens
RSKRSRLLHSDYMNMTPRRPGPTRKHYQPYAPPRDFAAYRS

SEQ ID NO: 50 - protein, 8 aa, Picornavirus
  VARIANT 2: note = X can either Valine or Isoleucine
  VARIANT 4: note = X can be any amino acid
DXEXNPGP

SEQ ID NO: 51 - protein, 21 aa, unidentified
MKSLRVLLVILWLQLSWVWSQ

SEQ ID NO: 52 - protein, 15 aa, unidentified
MLSLLLLLLGLGSVF

SEQ ID NO: 53 - protein, 19 aa, unidentified
MGPQLLGYVVLCLLGAGPL

SEQ ID NO: 54 - DNA, 1785 bp, unidentified
  source 1..1785: mol_type = other DNA
atgctgagcctgctgctgctgctgctgggcctgggaagcgtgttcagcgccgtgatcagccagaagccttcccgggacatctgccagagaggcaccagcctgacaatccagtgtcaggtggattcccaggtgaccatgatgttttggtacaggcagcagccaggccagtctctgaccctgatcgccacagccaaccagggctctgaggccacctatgagagcggcttcgtgatcgacaagtttcccatctcccgccctaacctgacattctctaccctgacagtgtccaatatgtctcccgaggacagctccatctacctgtgctccgtggagccaggctacgccgatacacagtattttggaccaggaaccaggctgacagtgctggaggatctacgtaacgtgacaccacccaaagtctcactgtttgagcctagcaaggcagaaattgccaacaagcagaaggccaccctggtgtgcctggcaagagggttctttccagatcacgtggagctgtcctggtgggtcaacggcaaagaagtgcattctggggtctgcaccgacccccaggcttacaaggagagtaattactcatattgtctgtcaagccggctgagagtgtccgccacattctggcacaaccctaggaatcatttccgctgccaggtccagtttcacggcctgagtgaggaagataaatggccagaggggtcacctaagccagtgacacagaacatcagcgcagaagcctggggacgagcagactgtggcattactagcgcctcctatcatcagggcgtgctgagcgccactatcctgtacgagattctgctgggaaaggccaccctgtatgctgtgctggtctccggcctggtgctgatggccatggtcaagaaaaagaactctgggagtggagccacaaatttctctctgctgaaacaggctggagatgtggaggaaaaccccggccctatgaagagcctgcgcgtgctgctggtcatcctgtggctgcaattgtcttgggtgtggagccaggaggaccaggtgacccagtccccagaggccctgaggctgcaggagggagagagctcctctctgaactgctcctacacagtgtctggcctgcggggcctgttctggtatagacaggatcctggcaagggcccagagttcctgtttaccctgtactctgccggcgaggagaaggagaaggagcggctgaaggccaccctgacaaagaaggagtctttcctgcacatcaccgcaccaaagcctgaggacagcgccacctacctgtgcgcagtgcaggcaagctccaacagcggctatgccctgaattttggcaagggcacctccctgctggtgacacctgatatccagaatccagagcccgccgtataccagctgaaggacccccgatctcaggatagtactctgtgcctgttcaccgactttgatagtcagatcaatgtgcctaaaaccatggaatccggaacttttattaccgacaagtgcgtgctggatatgaaagccatggacagtaagtcaaacggcgccatcgcttggagcaatcagacatccttcacttgccaggatatcttcaaggagaccaacgcaacatacccatcctctgacgtgccctgtgatgccaccctgacagagaagtctttcgaaacagacatgaacctgaattttcagaatctgagcgtgatgggcctgagaatcctgctgctgaaggtcgctgggtttaatctgctgatgacactgcggctgtggtcctcatga

SEQ ID NO: 55 - DNA, 1806 bp, unidentified
  source 1..1806: mol_type = other DNA
atgggaccacagctgctgggatacgtggtgctgtgcctgctgggagcaggaccactggaggcacaggtgacccagaacccaaggtatctgatcaccgtgacaggcaagaagctgaccgtgacatgttcccagaacatgaatcacgagtacatgtcttggtataggcaggaccctggcctgggcctgcgccagatctactatagcatgaatgtggaggtgaccgacaagggcgatgtgcctgagggctacaaggtgtcccggaaggagaagagaaacttcccactgatcctggagtctcccagccctaatcagacatctctgtacttttgcgccagctccctgtctagctcctataacgagcagttctttggaccaggaaccaggctgacagtgctggaggatctacgtaacgtgacaccacccaaagtctcactgtttgagcctagcaaggcagaaattgccaacaagcagaaggccaccctggtgtgcctggcaagagggttctttccagatcacgtggagctgtcctggtgggtcaacggcaaagaagtgcattctggggtctgcaccgacccccaggcttacaaggagagtaattactcatattgtctgtcaagccggctgagagtgtccgccacattctggcacaaccctaggaatcatttccgctgccaggtccagtttcacggcctgagtgaggaagataaatggccagaggggtcacctaagccagtgacacagaacatcagcgcagaagcctggggacgagcagactgtggcattactagcgcctcctatcatcagggcgtgctgagcgccactatcctgtacgagattctgctgggaaaggccaccctgtatgctgtgctggtctccggcctggtgctgatggccatggtcaagaaaaagaactctgggagtggagccacaaatttctctctgctgaaacaggctggagatgtggaggaaaaccccggccctatgaagagcctgcgcgtgctgctggtcatcctgtggctgcaattgtcttgggtgtggagccagtcccagcagggagaggaggacccacaggccctgagcatccaggagggcgagaacgccaccatgaattgctcttacaagacaagcatcaacaatctgcagtggtataggcagaactccggcaggggcctggtgcacctgatcctgatcaggtccaatgagcgcgagaagcactctggccggctgagagtgaccctggatacatctaagaagagctcctctctgctgatcaccgcaagcagggcagcagacacagcatcctacttctgtgccaccgatgcaggagcatattccggaggaggagcagacggcctgacctttggcaagggcacacacctgatcatccagcccgatatccagaaccccgagcctgccgtataccagctgaaggacccccgatctcaggatagtactctgtgcctgttcaccgactttgatagtcagatcaatgtgcctaaaaccatggaatccggaacttttattaccgacaagtgcgtgctggatatgaaagccatggacagtaagtcaaacggcgccatcgcttggagcaatcagacatccttcacttgccaggatatcttcaaggagaccaacgcaacatacccatcctctgacgtgccctgtgatgccaccctgacagagaagtctttcgaaacagacatgaacctgaattttcagaatctgagcgtgatgggcctgagaatcctgctgctgaaggtcgctgggtttaatctgctgatgacactgcggctgtggtcctcatga